European Patent Application EP 4 299 762 A1, published January 3, 2024. Title: Detection kit for oral cancer, use of reagent, reagent, detection device for oral cancer, information acquisition method and program. Applicant: Kagoshima University. The sequence listing filed with the application follows.

SEQUENCE LISTING (28 sequences)

SEQ ID NO: 1 - DNA, 52 bp, Artificial Sequence
  Probe for TP73
cgcccgcgaaggggacgcagcgaaaccggggcccgcgccaggccagccggga

SEQ ID NO: 2 - DNA, 64 bp, Artificial Sequence
  Probe for CASP8
ctttccaataaagcatgtccagcgctcgggctttagtttgcacgtccatgaattgtctgccaca

SEQ ID NO: 3 - DNA, 58 bp, Artificial Sequence
  Probe for VHL
gcgaagactacggaggtcgactcgggagcgcgcacgcagctccgccccgcgtccgacc

SEQ ID NO: 4 - DNA, 63 bp, Artificial Sequence
  Probe for RARB
agaaaacgccggcttgtgcgctcgctgcctgcctctctggctgtctgcttttgcagggctgct

SEQ ID NO: 5 - DNA, 61 bp, Artificial Sequence
  Probe 1 for MHL1
ctgctgaggtgatctggcgcagagcggaggaggtgcttggcgcttctcaggctcctcctct

SEQ ID NO: 6 - DNA, 67 bp, Artificial Sequence
  Probe 2 for MLH1
cgttgagcatctagacgtttccttggctcttctggcgccaaaatgtcgttcgtggcaggggttattc

SEQ ID NO: 7 - DNA, 49 bp, Artificial Sequence
  Probe 1 for RASSF1
ggccacagggcgggccccgacttcagcgcctcccccaggatccagactg

SEQ ID NO: 8 - DNA, 55 bp, Artificial Sequence
  Probe 2 for RASSF1
cccacagtccctgcacccaggtttccattgcgcggctctcctcagctccttcccg

SEQ ID NO: 9 - DNA, 52 bp, Artificial Sequence
  Probe for FHIT
cgcgggtctgggtttccacgcgcgtcaggtcatcaccccggagcccagtggg

SEQ ID NO: 10 - DNA, 59 bp, Artificial Sequence
  Probe for APC
cagctgtgtaatccgctggatgcggaccagggcgctccccattcccgtcgggagcccgc

SEQ ID NO: 11 - DNA, 55 bp, Artificial Sequence
  Probe for ESR1
agcccgccgtgtacaactaccccgagggcgccgcctacgagttcaacgccgcggc

SEQ ID NO: 12 - DNA, 75 bp, Artificial Sequence
  Probe for CDKN2A
ggggaagaggaaagaggaagaagcgctcagatgctccgcggctgtcgtgaaggttaaaaccgaaaataaaaatgg

SEQ ID NO: 13 - DNA, 67 bp, Artificial Sequence
  Probe for CDKN2B
gactagtggagaaggtgcgacagctcctggaagccggcgcggatcccaacggagtcaaccgtttcgg

SEQ ID NO: 14 - DNA, 55 bp, Artificial Sequence
  Probe for DAPK1
cgcgaggatctggagcgaactgctgcgcctcggtgggccgctcccttccctccct

SEQ ID NO: 15 - DNA, 52 bp, Artificial Sequence
  Probe 1 for KLLN
caccggagcgggcgcaggagaggcctgcggggtgcgtcccactcacagggat

SEQ ID NO: 16 - DNA, 61 bp, Artificial Sequence
  Probe 2 for KLLN
ctttcatttttagggcaaacgagccgagttaccggggaagcgagaggtggggcgctgcaag

SEQ ID NO: 17 - DNA, 62 bp, Artificial Sequence
  Probe for PTEN
ctctcaaacttccatcatggctgcagcttccgagaggagagaactgagcgcagtcgcgtccc

SEQ ID NO: 18 - DNA, 55 bp, Artificial Sequence
  Probe for CD44
ctcctttcgcccgcgccctccgttcgctccggacaccatggacaagttttggtgg

SEQ ID NO: 19 - DNA, 51 bp, Artificial Sequence
  Probe for GSTP1
gaagagcggccggcgccgtgactcagcactggggcggagcggggcgggacc

SEQ ID NO: 20 - DNA, 61 bp, Artificial Sequence
  Probe for ATM
gggaggaggcgagaggagtcgggatctgcgctgcagccaccgccgcggttgatactacttt

SEQ ID NO: 21 - DNA, 67 bp, Artificial Sequence
  Probe for CADM1
cctggagcccgagtccttgcacgccaggcgcccgggagaacactttttccttgatccggggaaagca

SEQ ID NO: 22 - DNA, 55 bp, Artificial Sequence
  Probe for CDKN1B
cagcccctgcgcgctcctagagctcgggccgtggctcgtcggggtctgtgtcttt

SEQ ID NO: 23 - DNA, 60 bp, Artificial Sequence
  Probe for CHFR
cgcgagagtaggcgcgtggagggcgctcggccatctttgatcctgaccaggcgacttcgt

SEQ ID NO: 24 - DNA, 69 bp, Artificial Sequence
  Probe for BRCA2
cgggagaagcgtgaggggacagatttgtgaccggcgcggtttttgtcagcttactccggccaaaaaaga

SEQ ID NO: 25 - DNA, 55 bp, Artificial Sequence
  Probe for CDH13
gttctgtgcgttctcctgtcccaggtagggaagaggggctgccgggcgcgctctg

SEQ ID NO: 26 - DNA, 54 bp, Artificial Sequence
  Probe for HIC1
cgctccagataagagtgtgcggaaagcgcggcggggctgagacgcgaccaggac

SEQ ID NO: 27 - DNA, 60 bp, Artificial Sequence
  Probe for BRCA1
ttctcagataactgggcccctgcgctcaggaggccttcaccctctgctctgggtaaaggt

SEQ ID NO: 28 - DNA, 52 bp, Artificial Sequence
  Probe for TIMP3
ccagcgccgaggcagcctcgctgcgccccatcccgtcccgccgggcactcgg